European Patent Specification EP 3 630 977 B1, published February 21, 2024. Title: Methods and Compositions for Generation of High Producer Cell Lines to Promote Unnatural Amino Acid-Containing Protein Production. Applicant: Ambrx, Inc Chen, Sigeng Lu, Yingchun Tian, Feng. The sequence listing filed with the application follows.

SEQUENCE LISTING (92 sequences)

SEQ ID NO: 1 - DNA, 19 bp, CHO
aggcactcgctcaacttct

SEQ ID NO: 2 - DNA, 19 bp, CHO
tgagtgtgaccggctgttg

SEQ ID NO: 3 - DNA, 19 bp, CHO
tttcatccagtatcgagct

SEQ ID NO: 4 - DNA, 19 bp, CHO
gaacaaattgtccatctcg

SEQ ID NO: 5 - DNA, 19 bp, CHO
atgctgtaagaacgggagt

SEQ ID NO: 6 - DNA, 19 bp, CHO
gaagccggtcaaaccacgt

SEQ ID NO: 7 - DNA, 19 bp, CHO
tcatggattggccagtaac

SEQ ID NO: 8 - DNA, 19 bp, CHO
ccactgggcgagacggtgc

SEQ ID NO: 9 - DNA, 19 bp, CHO
gaagcaccggtcctggatc

SEQ ID NO: 10 - DNA, 19 bp, CHO
agctctgtaggtggcgcac

SEQ ID NO: 11 - DNA, 19 bp, CHO
tgacatatgcctcggtaat

SEQ ID NO: 12 - DNA, 19 bp, CHO
taatcggtggaccccgaat

SEQ ID NO: 13 - DNA, 20 bp, CHO
aacaggagtatactctcttg

SEQ ID NO: 14 - DNA, 21 bp, CHO
cgccagacaaagcctatcgca

SEQ ID NO: 15 - DNA, 20 bp, CHO
agcctacgatcccaaggggg

SEQ ID NO: 16 - DNA, 19 bp, CHO
gcctcctcgatgtgcctgg

SEQ ID NO: 17 - DNA, 19 bp, CHO
cattgtccaggtccccctt

SEQ ID NO: 18 - DNA, 19 bp, CHO
acaatgcccgtcgtctgac

SEQ ID NO: 19 - DNA, 19 bp, CHO
tgaccctgttcatcagcgc

SEQ ID NO: 20 - DNA, 19 bp, CHO
tcagcgcggtccaggacca

SEQ ID NO: 21 - DNA, 19 bp, CHO
tccaggaccaggtggtgcc

SEQ ID NO: 22 - DNA, 19 bp, CHO
tcgatgagctgatgctttg

SEQ ID NO: 23 - DNA, 19 bp, CHO
agctgatgctttgggccga

SEQ ID NO: 24 - DNA, 19 bp, CHO
gaggactgccccgaagtcc

SEQ ID NO: 25 - DNA, 19 bp, CHO
ggcggtgttcgccgagatc

SEQ ID NO: 26 - DNA, 19 bp, CHO
ccgagatcggcccgcgcat

SEQ ID NO: 27 - DNA, 19 bp, CHO
gcgcatggccgagttgagc

SEQ ID NO: 28 - DNA, 19 bp, CHO
cagggcctcggccgagcct

SEQ ID NO: 29 - DNA, 19 bp, CHO
cccgctgccgcccccctgt

SEQ ID NO: 30 - DNA, 19 bp, CHO
ggcttggggatgccctgcg

SEQ ID NO: 31 - DNA, 19 bp, CHO
tacatcatcgcccagtgtg

SEQ ID NO: 32 - DNA, 19 bp, CHO
agcttcttcttgaattcgc

SEQ ID NO: 33 - DNA, 19 bp, CHO
atgaagacgaagagggtca

SEQ ID NO: 34 - DNA, 19 bp, CHO
agatgcccatattattggc

SEQ ID NO: 35 - DNA, 19 bp, CHO
atctggactcagacccctt

SEQ ID NO: 36 - DNA, 19 bp, CHO
gcaggcaatgcattggact

SEQ ID NO: 37 - DNA, 19 bp, CHO
ctctttttggcacgctcca

SEQ ID NO: 38 - DNA, 19 bp, CHO
atccacagtgaatttgtgc

SEQ ID NO: 39 - DNA, 19 bp, CHO
cgttttgcccgtttaagaa

SEQ ID NO: 40 - DNA, 20 bp, CHO
gcagatatgttattctccgc

SEQ ID NO: 41 - DNA, 20 bp, CHO
gatccgtccacaaccttggc

SEQ ID NO: 42 - DNA, 20 bp, CHO
gataaactgcaatctggttg

SEQ ID NO: 43 - DNA, 20 bp, CHO
agggttatgagcctccctag

SEQ ID NO: 44 - DNA, 20 bp, CHO
ggctaccatgtaaagagacc

SEQ ID NO: 45 - DNA, 19 bp, CHO
cagacagccttctcttgct

SEQ ID NO: 46 - DNA, 20 bp, CHO
agagctcctgagaggcatga

SEQ ID NO: 47 - DNA, 19 bp, CHO
tttcacgctgtgacaccca

SEQ ID NO: 48 - DNA, 20 bp, CHO
cagaaccacaccaagaattg

SEQ ID NO: 49 - DNA, 20 bp, CHO
tgtttaggaccttcggtttc

SEQ ID NO: 50 - DNA, 20 bp, CHO
atgtcaagggcactatagac

SEQ ID NO: 51 - DNA, 19 bp, CHO
cccaacgcaagagaccttc

SEQ ID NO: 52 - DNA, 20 bp, CHO
agagtgaacctcagcgcacg

SEQ ID NO: 53 - DNA, 20 bp, CHO
agtgaaagagagaggagagg

SEQ ID NO: 54 - DNA, 22 bp, CHO
gatgaagtgaagttgctctacc

SEQ ID NO: 55 - DNA, 20 bp, CHO
ctacgcaaggcacgaggttc

SEQ ID NO: 56 - DNA, 20 bp, CHO
ataagcctctgctactccag

SEQ ID NO: 57 - DNA, 21 bp, CHO
cacttgaacaaaggcatcaag

SEQ ID NO: 58 - DNA, 21 bp, CHO
tctcattgagaaggcatgtgc

SEQ ID NO: 59 - DNA, 20 bp, CHO
gggaattccaaataggaccc

SEQ ID NO: 60 - DNA, 20 bp, CHO
ctgctcgggaaggttatgtt

SEQ ID NO: 61 - DNA, 21 bp, CHO
atggccaagttgaccagtgcc

SEQ ID NO: 62 - DNA, 21 bp, CHO
tcagtcctgctcctcggccac

SEQ ID NO: 63 - DNA, 21 bp, CHO
atgaaaaagcctgaactcacc

SEQ ID NO: 64 - DNA, 21 bp, CHO
tcattcctctgccctcggacg

SEQ ID NO: 65 - DNA, 21 bp, CHO
atgaccgagtacaagcccacg

SEQ ID NO: 66 - DNA, 21 bp, CHO
agtccgtggcccgaacgccca

SEQ ID NO: 67 - DNA, 21 bp, CHO
ggcagcgcgtcagccccctgc

SEQ ID NO: 68 - DNA, 21 bp, CHO
tcagtgccagttttcttggct

SEQ ID NO: 69 - DNA, 21 bp, CHO
gctgagggggcagcaagctgc

SEQ ID NO: 70 - DNA, 21 bp, CHO
ctgcccagcccgaggaggcag

SEQ ID NO: 71 - DNA, 21 bp, CHO
atgaagctactcgagaactcc

SEQ ID NO: 72 - DNA, 21 bp, CHO
tttcatcctcaccaccctggc

SEQ ID NO: 73 - DNA, 21 bp, CHO
caggtgggctcacatctttgc

SEQ ID NO: 74 - DNA, 21 bp, CHO
tcacatacagatcactggaac

SEQ ID NO: 75 - DNA, 21 bp, CHO
tcatactgtgttgagtgggac

SEQ ID NO: 76 - DNA, 21 bp, CHO
ccacactagagagcccacaac

SEQ ID NO: 77 - DNA, 24 bp, CHO
atgccatcatatatcgtgagcatc

SEQ ID NO: 78 - DNA, 23 bp, CHO
aaacaagcttgttccctaactag

SEQ ID NO: 79 - DNA, 22 bp, CHO
aggagtgtagtgtagtgatgat

SEQ ID NO: 80 - DNA, 21 bp, CHO
atttgctctgctgccctaact

SEQ ID NO: 81 - DNA, 21 bp, CHO
tgacagcaatggactgttctc

SEQ ID NO: 82 - DNA, 22 bp, CHO
cagcttcaggatatgtagggta

SEQ ID NO: 83 - DNA, 24 bp, CHO
aggcactcgctcaacttcggtttt

SEQ ID NO: 84 - DNA, 24 bp, CHO
cgaagttgagcgagtgcctcggtg

SEQ ID NO: 85 - DNA, 24 bp, CHO
tgagtgtgaccggctgttggtttt

SEQ ID NO: 86 - DNA, 25 bp, CHO
caacagcgcctcacactcaccggtg

SEQ ID NO: 87 - DNA, 25 bp, CHO
tttcatccatgtatcgagctgtttt

SEQ ID NO: 88 - DNA, 25 bp, CHO
agctcgatactggatgaagacggtg

SEQ ID NO: 89 - DNA, 24 bp, CHO
gaacaaattgtccatctcggtttt

SEQ ID NO: 90 - DNA, 24 bp, CHO
cgagatggacaatttgttccggtg

SEQ ID NO: 91 - DNA, 24 bp, CHO
atgctgtaagaacgggagtgtttt

SEQ ID NO: 92 - DNA, 25 bp, CHO
cactcccgttcttacagcatcggtg